European Patent Specification EP 3 983 066 B1, published March 5, 2025. Title: Treatment of heart failure in human subjects. Applicant: Cardior Pharmaceuticals GmbH. The sequence listing filed with the application follows.

SEQUENCE LISTING (3 sequences)

SEQ ID NO: 1 - DNA, 16 bp, Artificial Sequence
  oligonucleotide
  misc_feature (1)..(16): at least one G or T is a bridged nucleotide building block
atggctgtagactgtt

SEQ ID NO: 2 - DNA, 16 bp, Artificial Sequence
  oligonucleotide
  misc_feature (2)..(2): bridged or morpholino nucleotide building block
  misc_feature (4)..(4): bridged or morpholino nucleotide building block
  misc_feature (6)..(6): bridged or morpholino nucleotide building block
  misc_feature (8)..(8): bridged or morpholino nucleotide building block
  misc_feature (10)..(10): bridged or morpholino nucleotide building block
  misc_feature (15)..(15): bridged or morpholino nucleotide building block
  misc_feature (16)..(16): bridged or morpholino nucleotide building block
atggctgtagactgtt

SEQ ID NO: 3 - DNA, 16 bp, Artificial Sequence
  oligonucleotide CDR132L
  misc_structure (1)..(1): 2'deoxyadenosine
  misc_feature (1)..(16): phosphorothioate linkage
  misc_feature (2)..(2): LNA building block
  misc_structure (3)..(3): 2'deoxyguanosine
  misc_feature (4)..(4): LNA building block
  misc_structure (5)..(5): 2'deoxycytidine
  misc_feature (6)..(6): LNA building block
  misc_structure (7)..(7): 2'deoxyguanosine
  misc_feature (8)..(8): LNA building block
  misc_structure (9)..(9): 2'deoxyadenosine
  misc_feature (10)..(10): LNA building block
  misc_structure (11)..(11): 2'deoxyadenosine
  misc_structure (12)..(12): 2'deoxycytidine
  misc_structure (13)..(13): thymidine
  misc_structure (14)..(14): 2'deoxyguanosine
  misc_feature (15)..(15): LNA building block
  misc_feature (16)..(16): LNA building block
atggctgtagactgtt